European Patent Application EP 4 752 152 A1, published June 3, 2026. Title: 甾类化合物、其制备方法和应用. Applicant: 珂阑（上海）医药科技有限公司. Application WO. The sequence listing filed with the application follows.

SEQUENCE LISTING (2 sequences)

SEQ ID NO: 1 - DNA, 23 bp, synthetic construct
  source 1..23: mol_type = other DNA
aaggacctgtctaggtttgatgc

SEQ ID NO: 2 - DNA, 21 bp, synthetic construct
  source 1..21: mol_type = other DNA
tggcttcataggtgacttcca